European Patent Specification EP 4 095 244 B1, published August 7, 2024. Title: Novel sugar phosphate isomerase/epimerase variant and a method for producing L-lysine using the same. Applicant: CJ CheilJedang Corporation. The sequence listing filed with the application follows.

SEQUENCE LISTING (10 sequences)

SEQ ID NO: 1 - protein, 337 aa, Artificial Sequence
  (A321V)_sugar phosphate isomerase/epimerase
MKLGLYNAIFHDRTLPEALAAIKAAGLTGIELNTGGFLPATHIPTIDDILVSDDARDEFLGIFEGTGVDIYGLNCNGNPLHPNKAIGDKHAEDIRRSIRLAERLGQNRVVTMSGLPGGEPGAKYTNWVVNAWNSAALDVLDYQWDIAAEFWRETDRFAADHGVKVALELHPQNIVFNSADVHKLIDLTGATHVGVELDASHLFWQQMDPIAVIDHLGELIFHAAAKDVRVNKEWAQLNGVLDNSFRRLDPSENRTNLGGDEWANEWPKNSAWDFVALGRGHDVAYWTEFLRALHRVDPNMLVNIEHEDVSLGREEGVNEAVKVLIEANKALEESLVS

SEQ ID NO: 2 - DNA, 1014 bp, Artificial Sequence
  (A321V)_NCgl0169
atgaaactcggtctctacaacgcgatcttccacgaccgcaccctgccagaagcgctcgcagccatcaaagctgcaggtctcaccggaattgaactcaacaccggcggatttttgcctgcaacccacatcccgaccatcgatgacatcctggtcagcgatgatgcccgcgatgaattcctcgggattttcgaaggcaccggcgtcgacatctacggccttaactgcaacggcaacccgcttcaccccaacaaggcgatcggggacaagcatgccgaagacattcgacgttccatccgcctcgcagagcgcctcggccaaaaccgtgtggtcaccatgtctggtcttcctggtggcgaaccaggcgcgaagtacaccaactgggttgtcaacgcgtggaactccgcagccttggatgtccttgattaccaatgggatatcgcagctgaattctggcgcgagaccgaccgcttcgccgcagatcacggcgtgaaagtggctcttgagctgcacccacagaacatcgtgttcaactccgctgacgtgcataagctcatcgatctcaccggcgccacccacgtgggcgtcgaactggatgcatcacacctgttctggcagcagatggacccaatcgctgtgattgatcacctcggcgagctcatcttccacgccgccgccaaagacgtgcgagttaataaggaatgggctcagctcaacggtgtgctggacaacagcttccgacgccttgacccatccgaaaaccgcaccaacttgggcggcgacgagtgggcgaatgaatggccaaagaactctgcttgggatttcgttgctctgggccgcggtcatgacgttgcttactggaccgaattcctccgcgcacttcaccgcgtcgatccaaacatgctggtcaacatcgaacacgaggatgtttcactcggtcgcgaagaaggcgtcaacgaagccgttaaggtgctgatcgaggccaacaaggcactcgaagagtccctggtttcttaa

SEQ ID NO: 3 - protein, 337 aa, Artificial Sequence
  (WT)_sugar phosphate isomerase/epimerase
MKLGLYNAIFHDRTLPEALAAIKAAGLTGIELNTGGFLPATHIPTIDDILVSDDARDEFLGIFEGTGVDIYGLNCNGNPLHPNKAIGDKHAEDIRRSIRLAERLGQNRVVTMSGLPGGEPGAKYTNWVVNAWNSAALDVLDYQWDIAAEFWRETDRFAADHGVKVALELHPQNIVFNSADVHKLIDLTGATHVGVELDASHLFWQQMDPIAVIDHLGELIFHAAAKDVRVNKEWAQLNGVLDNSFRRLDPSENRTNLGGDEWANEWPKNSAWDFVALGRGHDVAYWTEFLRALHRVDPNMLVNIEHEDVSLGREEGVNEAAKVLIEANKALEESLVS

SEQ ID NO: 4 - DNA, 1014 bp, Artificial Sequence
  (WT)_NCgl0169
atgaaactcggtctctacaacgcgatcttccacgaccgcaccctgccagaagcgctcgcagccatcaaagctgcaggtctcaccggaattgaactcaacaccggcggatttttgcctgcaacccacatcccgaccatcgatgacatcctggtcagcgatgatgcccgcgatgaattcctcgggattttcgaaggcaccggcgtcgacatctacggccttaactgcaacggcaacccgcttcaccccaacaaggcgatcggggacaagcatgccgaagacattcgacgttccatccgcctcgcagagcgcctcggccaaaaccgtgtggtcaccatgtctggtcttcctggtggcgaaccaggcgcgaagtacaccaactgggttgtcaacgcgtggaactccgcagccttggatgtccttgattaccaatgggatatcgcagctgaattctggcgcgagaccgaccgcttcgccgcagatcacggcgtgaaagtggctcttgagctgcacccacagaacatcgtgttcaactccgctgacgtgcataagctcatcgatctcaccggcgccacccacgtgggcgtcgaactggatgcatcacacctgttctggcagcagatggacccaatcgctgtgattgatcacctcggcgagctcatcttccacgccgccgccaaagacgtgcgagttaataaggaatgggctcagctcaacggtgtgctggacaacagcttccgacgccttgacccatccgaaaaccgcaccaacttgggcggcgacgagtgggcgaatgaatggccaaagaactctgcttgggatttcgttgctctgggccgcggtcatgacgttgcttactggaccgaattcctccgcgcacttcaccgcgtcgatccaaacatgctggtcaacatcgaacacgaggatgtttcactcggtcgcgaagaaggcgtcaacgaagccgctaaggtgctgatcgaggccaacaaggcactcgaagagtccctggtttcttaa

SEQ ID NO: 5 - DNA, 37 bp, Artificial Sequence
  NCgl0169_1F
tgaattcgagctcggtacccgcttcgccgcagatcac

SEQ ID NO: 6 - DNA, 33 bp, Artificial Sequence
  NCgl0169_2R
ctcgatcagcaccttaacggcttcgttgacgcc

SEQ ID NO: 7 - DNA, 33 bp, Artificial Sequence
  NCgl0169_3F
ggcgtcaacgaagccgttaaggtgctgatcgag

SEQ ID NO: 8 - DNA, 38 bp, Artificial Sequence
  NCgl0169_4R
gtcgactctagaggatccccgcgctcttcgtcaagtac

SEQ ID NO: 9 - DNA, 17 bp, Artificial Sequence
  NCgl0169_5F
ccaggcgcgaagtacac

SEQ ID NO: 10 - DNA, 17 bp, Artificial Sequence
  NCgl0169_6R
cgacggggagtgaccac